European Patent Specification EP 3 857 237 B1, published March 1, 2023. Title: Methods for Characterizing Disulfide Bonds. Applicant: Regeneron Pharmaceuticals, Inc. Wang, Shunhai. The sequence listing filed with the application follows.

SEQUENCE LISTING (4 sequences)

SEQ ID NO: 1 - protein, 14 aa, Artificial Sequence
  Peptide standard
THTCPPCPAPELLG

SEQ ID NO: 2 - protein, 4 aa, Artificial Sequence
  Peptide standard
CPTH

SEQ ID NO: 3 - protein, 10 aa, Artificial Sequence
  Peptide standard
PPCPAPELLG

SEQ ID NO: 4 - protein, 15 aa, Artificial Sequence
  Peptide standard
YGPPCPPCPAPEFLG